European Patent Application EP 4 198 044 A1, published June 21, 2023. Title: An isolated S. salivarius strain and its use as an antimicrobial producing probiotic. Applicant: Munster Technological University Teagasc, The Agriculture and Food Development Authority. The sequence listing filed with the application follows.

SEQUENCE LISTING (19 sequences)

SEQ ID NO: 1 - protein, 34 aa, Streptococcus salivarius
ITSYSLCTPGCKTGVLMACHLKTATCNCSIIVSK

SEQ ID NO: 2 - DNA, 174 bp, Streptococcus salivarius
atgagtacaaatgacttcaacttggatcttgtatctgtttcaaaatcaaatgcaggtgcttcaactcgtattacaagttattcgctatgtacaccgggatgtaaaactggtgtattaatggcgtgtcatcttaaaactgctacatgtaactgtagtatcattgtttcaaaataa

SEQ ID NO: 3 - protein, 57 aa, Streptococcus salivarius
MSTNDFNLDLVSVSKSNAGASTRITSYSLCTPGCKTGVLMACHLKTATCNCSIIVSK

SEQ ID NO: 4 - DNA, 1347 bp, Streptococcus salivarius
tttatttgaaaggggcaattgctccactacaagatggacctgcgttgtattagctagtaggtgaggtaacggctcacctaggcgacgatacatagccgacctgagagggtgatcggccacactgggactgagacacggcccagactcctacgggaggcagcagtagggaatcttcggcaatgggggcaaccctgaccgagcaacgccgcgtgagtgaagaaggttttcggatcgtaaagctctgttgtaagtcaagaacgagtgtgagagtggaaagttcacactgtgacggtagcttaccagaaagggacggctaactacgtgccagcagccgcggtaatacgtaggtcccgagcgttgtccggatttattgggcgtaaagcgagcgcaggcggtttgataagtctgaagttaaaggctgtggctcaaccatagttcgctttggaaactgtcaaacttgagtgcagaaggggagagtggaattccatgtgtagcggtgaaatgcgtagatatatggaggaacaccggtggcgaaagcggctctctggtctgtaactgacgctgaggctcgaaagcgtggggagcgaacaggattagataccctggtagtccacgccgtaaacgatgagtgctaggtgttggatcctttccgggattcagtgccgcagctaacgcattaagcactccgcctggggagtacgaccgcaaggttgaaactcaaaggaattgacgggggcccgcacaagcggtggagcatgtggtttaattcgaagcaacgcgaagaaccttaccaggtcttgacatcccgatgctatttctagagatagaaagttacttcggtacatcggtgacaggtggtgcatggttgtcgtcagctcgtgtcgtgagatgttgggttaagtcccgcaacgagcgcaacccctattgttagttgccatcattcagttgggcactctagcgagactgccggtaataaaccggaggaaggtggggatgacgtcaaatcatcatgccccttatgacctgggctacacacgtgctacaatggttggtacaacgagttgcgagtcggtgacggcaagctaatctcttaaagccaatctcagttcggattgtaggctgcaactcgcctacatgaagtcggaatcgctagtaatcgcggatcagcacgccgcggtgaatacgttcccgggccttgtacacaccgcccgtcacaccacgagagtttgtaacacccgaagtcggtgaggtaaccttttggagccagccgcctaaggtgggatagatgattggggtgaagtcgtaacaaggtagccgtatcggaaggtgcggctggatcacctcctt

SEQ ID NO: 5 - DNA, 20 bp, Artificial Sequence
  mefE forward primer
ccatcgacgtattgggtgct

SEQ ID NO: 6 - DNA, 20 bp, Artificial Sequence
  mefE reverse primer
aaacggctaaactggtcccc

SEQ ID NO: 7 - protein, 34 aa, Lactococcus lactis
ITSISLCTPGCKTGALMGCNMKTATCHCSIHVSK

SEQ ID NO: 8 - protein, 34 aa, Lactococcus lactis
ITSISLCTPGCKTGALMGCNMKTATCNCSIHVSK

SEQ ID NO: 9 - protein, 34 aa, Lactococcus lactis
ITSISLCTPGCKTGALMGCNMKTATCNCSVHVSK

SEQ ID NO: 10 - protein, 34 aa, Lactococcus lactis
ITSISLCTPGCKTGVLMGCNLKTATCNCSVHVSK

SEQ ID NO: 11 - protein, 34 aa, Streptococcus hyointestinalis
FTSISMCTPGCKTGALMTCNYKTATCHCSIKVSK

SEQ ID NO: 12 - protein, 35 aa, Staphylococcus capitis
ITSKSLCTPGCKTGALQTCFAKTATCHCSGHVHTK

SEQ ID NO: 13 - protein, 31 aa, Streptococcus uberis
ITSKSLCTPGCKTGILMTCPLKTATCGCHFG

SEQ ID NO: 14 - protein, 31 aa, Streptococcus uberis
VTSKSLCTPGCKTGILMTCPLKTATCGCHFG

SEQ ID NO: 15 - protein, 31 aa, Streptococcus gallolyticus
VTSKSLCTPGCKTGILMTCAIKTATCGCHFG

SEQ ID NO: 16 - protein, 39 aa, APILACTOBACILLUS KUNKEEI
ITSYVLCTPGCITGRLMGCNNKTKTCHCHSSNHFSFHAR

SEQ ID NO: 17 - protein, 33 aa, BLAUTIA OBEUM
YKSKSACTPGCPTGILMTCPLKTATCGCHITGK

SEQ ID NO: 18 - protein, 34 aa, Streptococcus salivarius
FTSHSLCTPGCITGVLMGCHIQSIGCNVHIHISK

SEQ ID NO: 19 - protein, 32 aa, BLAUTIA OBEUM
TSQHSFCTPNCLTGFLCPPKTQLTCTCKLKGQ